European Patent Specification EP 3 464 342 B1, published March 18, 2026. Title: Mutant light-inducible ion channels. Applicant: Max-Planck-Gesellschaft zur Förderung der Wissenschaften e.V. The sequence listing filed with the application follows.

SEQUENCE LISTING (10 sequences)

SEQ ID NO: 1 - protein, 349 aa, Artificial
  Chrimson derived from Chlamydomonas noctigama
MAELISSATRSLFAAGGINPWPNPYHHEDMGCGGMTPTGECFSTEWWCDPSYGLSDAGYGYCFVEATGGYLVVGVEKKQAWLHSRGTPGEKIGAQVCQWIAFSIAIALLTFYGFSAWKATCGWEEVYVCCVEVLFVTLEIFKEFSSPATVYLSTGNHAYCLRYFEWLLSCPVILIKLSNLSGLKNDYSKRTMGLIVSCVGMIVFGMAAGLATDWLKWLLYIVSCIYGGYMYFQAAKCYVEANHSVPKGHCRMVVKLMAYAYFASWGSYPILWAVGPEGLLKLSPYANSIGHSICDIIAKEFWTFLAHHLRIKIHEHILIHGDIRKTTKEIGGEEVEVEEFVEEEDEDTV

SEQ ID NO: 2 - protein, 345 aa, Artificial
  CsChrimson
MSRLVAASWLLALLLCGITSTTTASSAPAASSTDGTAAAAVSHYAMNGFDELAKGAVVPEDHFVCGPADKCYCSAWLHSRGTPGEKIGAQVCQWIAFSIAIALLTFYGFSAWKATCGWEEVYVCCVEVLFVTLEIFKEFSSPATVYLSTGNHAYCLRYFEWLLSCPVILIKLSNLSGLKNDYSKRTMGLIVSCVGMIVFGMAAGLATDWLKWLLYIVSCIYGGYMYFQAAKCYVEANHSVPKGHCRMVVKLMAYAYFASWGSYPILWAVGPEGLLKLSPYANSIGHSICDIIAKEFWTFLAHHLRIKIHEHILIHGDIRKTTKMEIGGEEVEVEEFVEEEDEDTV

SEQ ID NO: 3 - protein, 25 aa, Artificial
  Helix 6 consensus motif
  VARIANT (12)..(12): wherein Xaa12 is Phe or Tyr, in particular wherein Xaa12 is Phe
  VARIANT (18)..(18): wherein Xaa18 is Met or Ser, in particular wherein Xaa18 is Met
  VARIANT (19)..(19): wherein Xaa19 is Phe or Tyr, in particular wherein Xaa19 is Phe
CRMVVKLMAYAXFASWGXXPILWAV

SEQ ID NO: 4 - protein, 9 aa, Artificial
  Retinal binding site consensus motif
  VARIANT (1)..(1): wherein Xaa1 is Leu, Ile, Ala, or Cys
  VARIANT (3)..(5): wherein Xaa3, Xaa4, and Xaa5 is independently any amino acid
  VARIANT (7)..(8): wherein Xaa7 and Xaa8 is independently any amino acid
  VARIANT (9)..(9): wherein Xaa9 is Thr, Phe, or Tyr
XDXXXKXXX

SEQ ID NO: 5 - protein, 315 aa, Chlamydomonas reinhardtii
MDYGGALSAVGRELLFVTNPVVVNGSVLVPEDQCYCAGWIESRGTNGAQTASNVLQWLAAGFSILLLMFYAYQTWKSTCGWEEIYVCAIEMVKVILEFFFEFKNPSMLYLATGHRVQWLRYAEWLLTCPVILIHLSNLTGLSNDYSRRTMGLLVSDIGTIVWGATSAMATGYVKVIFFCLGLCYGANTFFHAAKAYIEGYHTVPKGRCRQVVTGMAWLFFVSWGMFPILFILGPEGFGVLSVYGSTVGHTIIDLMSKNCWGLLGHYLRVLIHEHILIHGDIRKTTKLNIGGTEIEVETLVEDEAEAGAVNKGTGK

SEQ ID NO: 6 - protein, 300 aa, Volvox carteri
MDYPVARSLIVRYPTDLGNGTVCMPRGQCYCEGWLRSRGTSIEKTIAITLQWVVFALSVACLGWYAYQAWRATCGWEEVYVALIEMMKSIIEAFHEFDSPATLWLSSGNGVVWMRYGEWLLTCPVLLIHLSNLTGLKDDYSKRTMGLLVSDVGCIVWGATSAMCTGWTKILFFLISLSYGMYTYFHAAKVYIEAFHTVPKGICRELVRVMAWTFFVAWGMFPVLFLLGTEGFGHISPYGSAIGHSILDLIAKNMWGVLGNYLRVKIHEHILLYGDIRKKQKITIAGQEMEVETLVAEEED

SEQ ID NO: 7 - protein, 352 aa, Artificial
  ReaChR
MVSRRPWLLALALAVALAAGSAGASTGSDATVPVATQDGPDYVFHRAHERMLFQTSYTLENNGSVICIPNNGQCFCLAWLKSNGTNAEKLAANILQWVVFALSVACLGWYAYQAWRATCGWEEVYVALIEMMKSIIEAFHEFDSPATLWLSSGNGVVWMRYGEWLLTCPVILIHLSNLTGLKDDYSKRTMGLLVSDVGCIVWGATSAMCTGWTKILFFLISLSYGMYTYFHAAKVYIEAFHTVPKGLCRQLVRAMAWLFFVSWGMFPVLFLLGPEGFGHISPYGSAIGHSILDLIAKNMWGVLGNYLRVKIHEHILLYGDIRKKQKITIAGQEMEVETLVAEEEDKYESSLE

SEQ ID NO: 8 - protein, 315 aa, Artificial
  ChR2 helix 6 swap mutant
MDYGGALSAVGRELLFVTNPVVVNGSVLVPEDQCYCAGWIESRGTNGAQTASNVLQWLAAGFSILLLMFYAYQTWKSTCGWEEIYVCAIEMVKVILEFFFEFKNPSMLYLATGHRVQWLRYAEWLLTCPVILIHLSNLTGLSNDYSRRTMGLLVSDIGTIVWGATSAMATGYVKVIFFCLGLCYGANTFFHAAKAYIEGYHTVPKGRCRMVVKLMAYAYFASWGSYPILWAVGPEGFGVLSVYGSTVGHTIIDLMSKNCWGLLGHYLRVLIHEHILIHGDIRKTTKLNIGGTEIEVETLVEDEAEAGAVNKGTGK

SEQ ID NO: 9 - protein, 300 aa, Artificial
  VChR1 helix 6 swap mutant
MDYPVARSLIVRYPTDLGNGTVCMPRGQCYCEGWLRSRGTSIEKTIAITLQWVVFALSVACLGWYAYQAWRATCGWEEVYVALIEMMKSIIEAFHEFDSPATLWLSSGNGVVWMRYGEWLLTCPVLLIHLSNLTGLKDDYSKRTMGLLVSDVGCIVWGATSAMCTGWTKILFFLISLSYGMYTYFHAAKVYIEAFHTVPKGICRMVVKLMAYAYFASWGSYPILWAVGTEGFGHISPYGSAIGHSILDLIAKNMWGVLGNYLRVKIHEHILLYGDIRKKQKITIAGQEMEVETLVAEEED

SEQ ID NO: 10 - protein, 352 aa, Artificial
  ReaChR helix 6 swap mutant
MVSRRPWLLALALAVALAAGSAGASTGSDATVPVATQDGPDYVFHRAHERMLFQTSYTLENNGSVICIPNNGQCFCLAWLKSNGTNAEKLAANILQWVVFALSVACLGWYAYQAWRATCGWEEVYVALIEMMKSIIEAFHEFDSPATLWLSSGNGVVWMRYGEWLLTCPVILIHLSNLTGLKDDYSKRTMGLLVSDVGCIVWGATSAMCTGWTKILFFLISLSYGMYTYFHAAKVYIEAFHTVPKGLCRMVVKLMAYAYFASWGSYPILWAVGPEGFGHISPYGSAIGHSILDLIAKNMWGVLGNYLRVKIHEHILLYGDIRKKQKITIAGQEMEVETLVAEEEDKYESSLE